European Patent Specification EP 3 180 419 B1, published June 4, 2025. Title: MUTATIONS IN IRON-SULFUR CLUSTER PROTEINS THAT IMPROVE XYLOSE UTILIZATION. Applicant: MASCOMA CORPORATION Froehlich, Allan Henningsen, Brooks Covalla, Sean. The sequence listing filed with the application follows.

SEQUENCE LISTING (42 sequences)

SEQ ID NO: 1 - protein, 436 aa, Artificial Sequence
  Chimeric Xylose Isomerase 1
MSELFQNIPKIKYEGANSKNPLAFHYYDAEKEIMGKKMKDWLRFAMAWWHTLCAEGSDQFGPGTKTFPWNEGTDPIEKAKQKVDAGFEIMTKLGIEHYCFHDVDLVDEGKNVEEYEKNLKTIVAYLKEKQKETGIKLLWGTANVFGHARYMNGAATNPDFDVVARAAVQIKNAIDATIELGGENYVFWGGREGYMSLLNTNMKREKDHLAMMLTMARDYGRKNGFKGTFLIEPKPMEPTKHQYDVDSETVIGFLRHYGLDKDFALNIEVNHATLAGHTFEHELQAAADAGMLCSIDANRGDYQNGWDTDQFPMDIYELAQAWLVILEGGGLTTGGTNFDAKTRRNSTDLEDIFIAHIGGMDAFARALMIAADILENSDYRKMRAERYASFDAGEGKAFEDGKLTLEDLRTIALRDGEPKQISGKQELYEMIVNLHI

SEQ ID NO: 2 - DNA, 1311 bp, Artificial Sequence
  Chimeric Xylose Isomerase 1
atgtctgaattgttccaaaacatcccaaagatcaagtacgaaggtgctaactctaagaacccattggctttccactactacgacgctgaaaaggaaatcatgggtaagaagatgaaggactggttgagattcgctatggcttggtggcacactttgtgtgctgaaggttctgaccaattcggtccaggtactaagactttcccatggaacgaaggtactgacccaatcgaaaaggctaagcaaaaggttgacgctggtttcgaaatcatgactaagttgggtatcgaacactactgtttccacgacgttgacttggttgacgaaggtaagaacgttgaagaatacgaaaagaacttgaagactatcgttgcttacttgaaggaaaagcaaaaggaaactggtatcaagttgttgtggggtactgctaacgttttcggtcacgctagatacatgaacggtgctgctactaacccagacttcgacgttgttgccagagctgctgttcaaattaagaacgctattgacgctactattgaattgggtggtgaaaactacgttttctggggtggtagagaaggttacatgtctttgttgaacaccaacatgaagagagaaaaggatcatttggccatgatgttgactatggctagagattacggtagaaagaatggtttcaagggtactttcttgatcgaacctaaacctatggaacctactaagcaccaatacgatgttgattccgaaaccgttatcggtttcttgagacattacggtttggataaggatttcgccttgaacatcgaagttaaccatgctactttggctggtcatactttcgaacatgaattgcaagctgctgctgatgctggtatgttgtgttctattgatgctaacagaggtgactaccaaaatggttgggatactgatcaattcccaatggatatctacgaattggctcaagcttggttggttattttggaaggtggtggtttgactactggtggtactaattttgatgccaagaccagaagaaactccactgatttggaagacatcttcattgcccatatcggtggtatggatgcttttgctagagctttgatgattgctgccgatattttggaaaactccgactacagaaagatgagagctgaaagatacgcttcttttgatgctggtgaaggtaaggctttcgaagatggtaaattgaccttggaagatttgagaaccattgctttgagagatggtgaacctaagcaaatttccggtaagcaagaattatacgaaatgatcgtcaacttgcacatctaa

SEQ ID NO: 3 - protein, 438 aa, Artificial Sequence
  Chimeric Xylose Isomerase 2
MAKEYFPFTGKIPFEGKDSKNVMAFHYYEPEKVVMGKKMKDWLKFAMAWWHTLGGASADQFGGQTRSYEWDKAADAVQRAKDKMDAGFEIMDKLGIEYFCFHDVDLVEEGETIAEYERRMKEITDYALVKMKEYPNIKLLWGTANVFGHARYMNGAATNPDFDVVARAAVQIKNAIDATIELGGENYVFWGGREGYMSLLNTNMKREKDHLAMMLTMARDYGRKNGFKGTFLIEPKPMEPTKHQYDVDSETVIGFLRHYGLDKDFALNIEVNHATLAGHTFEHELQAAADAGMLCSIDANRGDYQNGWDTDQFPMDIYELAQAWLVILEGGGLTTGGTNFDAKTRRNSTDLEDIFIAHIGGMDAFARALMIAADILENSDYRKMRAERYASFDAGEGKAFEDGKLTLEDLRTIALRDGEPKQISGKQELYEMIVNLHI

SEQ ID NO: 4 - DNA, 1317 bp, Artificial Sequence
  Chimeric Xylose Isomerase 2
atggctaaggaatacttcccattcactggtaagatcccattcgaaggtaaggactctaagaacgttatggctttccactactacgaaccagaaaaggttgttatgggtaagaagatgaaggactggttgaagttcgctatggcttggtggcacactttgggtggtgcttctgctgaccaattcggtggtcaaactagatcttacgaatgggacaaggctgctgacgctgttcaaagagctaaggacaagatggacgctggtttcgaaatcatggacaagttgggtatcgaatacttctgtttccacgacgttgacttggttgaagaaggtgaaactatcgctgaatacgaaagaagaatgaaggaaatcactgactacgctttggttaagatgaaggaatacccaaacatcaagttgttgtggggtactgctaacgttttcggtcacgctagatacatgaacggtgctgctactaacccagacttcgacgttgttgccagagctgctgttcaaattaagaacgctattgacgctactattgaattgggtggtgaaaactacgttttctggggtggtagagaaggttacatgtctttgttgaacaccaacatgaagagagaaaaggatcatttggccatgatgttgactatggctagagattacggtagaaagaatggtttcaagggtactttcttgatcgaacctaaacctatggaacctactaagcaccaatacgatgttgattccgaaaccgttatcggtttcttgagacattacggtttggataaggatttcgccttgaacatcgaagttaaccatgctactttggctggtcatactttcgaacatgaattgcaagctgctgctgatgctggtatgttgtgttctattgatgctaacagaggtgactaccaaaatggttgggatactgatcaattcccaatggatatctacgaattggctcaagcttggttggttattttggaaggtggtggtttgactactggtggtactaattttgatgccaagaccagaagaaactccactgatttggaagacatcttcattgcccatatcggtggtatggatgcttttgctagagctttgatgattgctgccgatattttggaaaactccgactacagaaagatgagagctgaaagatacgcttcttttgatgctggtgaaggtaaggctttcgaagatggtaaattgaccttggaagatttgagaaccattgctttgagagatggtgaacctaagcaaatttccggtaagcaagaattatacgaaatgatcgtcaacttgcacatctaa

SEQ ID NO: 5 - protein, 437 aa, Artificial Sequence
  Chimeric Xylose Isomerase 3
MVKEYFPAIQKIKFEGKDSKNPMAFHYYDAEKEIMGKKMKDWLRFAMAWWHTLCAEGSDQFGPGTKTFPWNEGTDPIEKAKQKVDAGFEIMTKLGIEHYCFHDVDLVDEGKNVEEYEKNLKTIVAYLKEKQKETGIKLLWSTANVFGHKRYMNGAATNPYFPTVACVGTQIKNAIDACIALGGENYVFWGGREGYMSLLNTNMKREKDHLAMMLTMARDYGRKNGFKGTFLIEPKPMEPTKHQYDVDSETVIGFLRHYGLDKDFALNIEVNHATLAGHTFEHELQAAADAGMLCSIDANRGDYQNGWDTDQFPMDIYELAQAWLVILEGGGLTTGGTNFDAKTRRNSTDLEDIFIAHIGGMDAFARALMIAADILENSDYRKMRAERYASFDAGEGKAFEDGKLTLEDLRTIALRDGEPKQISGKQELYEMIVNLHI

SEQ ID NO: 6 - DNA, 1314 bp, Artificial Sequence
  Chimeric Xylose Isomerase 3
atggttaaggaatacttcccagctatccaaaagatcaagttcgaaggtaaggactctaagaacccaatggctttccactactacgacgctgaaaaggaaatcatgggtaagaagatgaaggactggttgagattcgctatggcttggtggcacactttgtgtgctgaaggttctgaccaattcggtccaggtactaagactttcccatggaacgaaggtactgacccaatcgaaaaggctaagcaaaaggttgacgctggtttcgaaatcatgactaagttgggtatcgaacactactgtttccacgacgttgacttggttgacgaaggtaagaacgttgaagaatacgaaaagaacttgaagactatcgttgcttacttgaaggaaaagcaaaaggaaactggtatcaagttgttgtggtctactgctaacgttttcggtcacaagagatatatgaacggtgctgctactaatccatactttccaactgttgcttgcgttggtactcaaatcaagaatgctattgatgcttgcattgctttgggtggtgaaaattatgttttctggggtggtagagaaggttacatgtctttgttgaacaccaacatgaagagagaaaaggatcatttggccatgatgttgactatggctagagattacggtagaaagaatggtttcaagggtactttcttgatcgaacctaaacctatggaacctactaagcaccaatacgatgttgattccgaaaccgttatcggtttcttgagacattacggtttggataaggatttcgccttgaacatcgaagttaaccatgctactttggctggtcatactttcgaacatgaattgcaagctgctgctgatgctggtatgttgtgttctattgatgctaacagaggtgactaccaaaatggttgggatactgatcaattcccaatggatatctacgaattggctcaagcttggttggttattttggaaggtggtggtttgactactggtggtactaattttgatgccaagaccagaagaaactccactgatttggaagacatcttcattgcccatatcggtggtatggatgcttttgctagagctttgatgattgctgccgatattttggaaaactccgactacagaaagatgagagctgaaagatacgcttcttttgatgctggtgaaggtaaggctttcgaagatggtaaattgaccttggaagatttgagaaccattgctttgagagatggtgaacctaagcaaatttccggtaagcaagaattatacgaaatgatcgtcaacttgcacatctaa

SEQ ID NO: 7 - protein, 438 aa, Artificial Sequence
  Directed Chimeric Xylose Isomerase 1
MAKEYFPFTGKIPFEGKDSKNVMAFHYYEPEKVVMGKKMKDWLKFAMAWWHTLGGASADQFGGQTRSYEWDKAADAVQRAKDKMDAGFEIMDKLGIEYFCFHDVDLVEEGETIAEYERRMKEITDYALVKMKEYPNIKLLWGTANVFGNKRYANGASTNPDFDVVARAIVQIKNAIDATIKLGGTNYVFWGGREGYMTLLNTDMKREQEHLARFLTMAKDYARKQGFTGTFFIEPKPCEPTKHQYDYDAATVIGFLRHFGLDKDFKLNLEVNHATLAGHTFEHELACAVDAGMLGSIDANRGDYQNGWDTDQFPIDQYELVQAWMEIIRGGGFTTGGTNFDAKTRRNSTDLEDIIIAHISGMDAMARALENAAKLLTESPYKKMKADRYASFDSGMGKDFEDGKLTFEQVYEYGKKVNEPKQTSGKQELYEAIVAMYM

SEQ ID NO: 8 - DNA, 1317 bp, Artificial Sequence
  Directed Chimeric Xylose Isomerase 1
atggctaaggaatacttcccattcactggtaagatcccattcgaaggtaaggactctaagaacgttatggctttccactactacgaaccagaaaaggttgttatgggtaagaagatgaaggactggttgaagttcgctatggcttggtggcacactttgggtggtgcttctgctgaccaattcggtggtcaaactagatcttacgaatgggacaaggctgctgacgctgttcaaagagctaaggacaagatggacgctggtttcgaaatcatggacaagttgggtatcgaatacttctgtttccacgacgttgacttggttgaagaaggtgaaactatcgctgaatacgaaagaagaatgaaggaaatcactgactacgctttggttaagatgaaggaatacccaaacatcaagttgttgtggggtactgctaacgttttcggtaacaagagatacgctaacggtgcttctactaacccagacttcgacgttgttgctagagctatcgttcaaatcaagaacgctatcgacgctactatcaagttgggtggtactaactacgttttctggggtggtagagaaggttacatgactttgttgaacaccgacatgaagagagaacaagaacatttggctagattcttgaccatggctaaagattacgctagaaagcaaggtttcaccggtacttttttcattgaacctaagccatgcgaacctaccaaacatcaatatgattacgatgctgccaccgttattggttttttgagacatttcggtttggacaaggacttcaagttgaacttggaagttaaccatgctactttggctggtcacactttcgaacacgaattggcttgtgctgttgacgctggtatgttgggttctatcgacgctaacagaggtgactaccaaaacggttgggacactgaccaattcccaatcgaccaatacgaattggttcaagcttggatggaaatcatcagaggtggtggtttcactactggtggtactaacttcgacgctaagactagaagaaactctactgacttggaagacatcatcatcgctcacatctctggtatggacgctatggctagagctttggaaaacgctgctaagttgttgactgaatctccatacaagaagatgaaggctgacagatacgcttctttcgactctggtatgggtaaggacttcgaagacggtaagttgactttcgaacaagtttacgaatacggtaagaaggttaacgaaccaaagcaaacttctggtaagcaagaattgtacgaagctatcgttgctatgtacatgtga

SEQ ID NO: 9 - protein, 443 aa, Artificial Sequence
  Directed Chimeric Xylose Isomerase 2
MKLTVGDKEYFKGIKPIKFEGKDSKNVMAFHYYEPEKVVMGKKMKDWLKFAMAWWHTLGGASADQFGGQTRSYEWDKAADAVQRAKDKMDAGFEIMDKLGIEYFCFHDVDLVEEGETIAEYERRMKEITDYALVKMKEYPNIKLLWGTANVFGNKRYANGASTNPDFDVVARAIVQIKNAIDATIKLGGTNYVFWGGREGYMTLLNTDMKREQEHLARFLTMAKDYARKQGFTGTFFIEPKPCEPTKHQYDYDAATVIGFLRHFGLDKDFKLNLEVNHATLAGHTFEHELACAVDAGMLGSIDANRGDYQNGWDTDQFPIDQYELVQAWMEIIRGGGFTTGGTNFDAKTRRNSTDLEDIIIAHISGMDAMARALENAAKLLTESPYKKMKADRYASFDSGMGKDFEDGKLTFEQVYEYGKKVNEPKQTSGKQELYEAIVAMYM

SEQ ID NO: 10 - DNA, 1332 bp, Artificial Sequence
  Directed Chimeric Xylose Isomerase 2
atgaagttgaccgttggtgacaaagaatacttcaagggtattaagccaatcaagttcgaaggtaaggactctaagaacgttatggctttccactactacgaaccagaaaaggttgttatgggtaagaagatgaaggactggttgaagttcgctatggcttggtggcacactttgggtggtgcttctgctgaccaattcggtggtcaaactagatcttacgaatgggacaaggctgctgacgctgttcaaagagctaaggacaagatggacgctggtttcgaaatcatggacaagttgggtatcgaatacttctgtttccacgacgttgacttggttgaagaaggtgaaactatcgctgaatacgaaagaagaatgaaggaaatcactgactacgctttggttaagatgaaggaatacccaaacatcaagttgttgtggggtactgctaacgttttcggtaacaagagatacgctaacggtgcttctactaacccagacttcgacgttgttgctagagctatcgttcaaatcaagaacgctatcgacgctactatcaagttgggtggtactaactacgttttctggggtggtagagaaggttacatgactttgttgaacaccgacatgaagagagaacaagaacatttggctagattcttgaccatggctaaagattacgctagaaagcaaggtttcaccggtacttttttcattgaacctaagccatgcgaacctaccaaacatcaatatgattacgatgctgccaccgttattggttttttgagacatttcggtttggacaaggacttcaagttgaacttggaagttaaccatgctactttggctggtcacactttcgaacacgaattggcttgtgctgttgacgctggtatgttgggttctatcgacgctaacagaggtgactaccaaaacggttgggacactgaccaattcccaatcgaccaatacgaattggttcaagcttggatggaaatcatcagaggtggtggtttcactactggtggtactaacttcgacgctaagactagaagaaactctactgacttggaagacatcatcatcgctcacatctctggtatggacgctatggctagagctttggaaaacgctgctaagttgttgactgaatctccatacaagaagatgaaggctgacagatacgcttctttcgactctggtatgggtaaggacttcgaagacggtaagttgactttcgaacaagtttacgaatacggtaagaaggttaacgaaccaaagcaaacttctggtaagcaagaattgtacgaagctatcgttgctatgtacatgtga

SEQ ID NO: 11 - protein, 438 aa, Bacteroides thetaiotaomicron
MATKEFFPGIEKIKFEGKDSKNPMAFRYYDAEKVINGKKMKDWLRFAMAWWHTLCAEGGDQFGGGTKQFPWNGNADAIQAAKDKMDAGFEFMQKMGIEYYCFHDVDLVSEGASVEEYEANLKEIVAYAKQKQAETGIKLLWGTANVFGHARYMNGAATNPDFDVVARAAVQIKNAIDATIELGGENYVFWGGREGYMSLLNTDQKREKEHLAQMLTIARDYARARGFKGTFLIEPKPMEPTKHQYDVDTETVIGFLKAHGLDKDFKVNIEVNHATLAGHTFEHELAVAVDNGMLGSIDANRGDYQNGWDTDQFPIDNYELTQAMMQIIRNGGLGTGGTNFDAKTRRNSTDLEDIFIAHIAGMDAMARALESAAALLDESPYKKMLADRYASFDGGKGKEFEDGKLTLEDVVAYAKTKGEPKQTSGKQELYEAILNMYC

SEQ ID NO: 12 - DNA, 1317 bp, Bacteroides thetaiotaomicron
atggcaacaaaagaattttttccgggaattgaaaagattaaatttgaaggtaaagatagtaagaacccgatggcattccgttattacgatgcagagaaggtgattaatggtaaaaagatgaaggattggctgagattcgctatggcatggtggcacacattgtgcgctgaaggtggtgatcagttcggtggcggaacaaagcaattcccatggaatggtaatgcagatgctatacaggcagcaaaagataagatggatgcaggatttgaattcatgcagaagatgggtatcgaatactattgcttccatgacgtagacttggtttcggaaggtgccagtgtagaagaatacgaagctaacctgaaagaaatcgtagcttatgcaaaacagaaacaggcagaaaccggtatcaaactactgtggggtactgctaatgtattcggtcacgcccgctatatgaacggtgcagctaccaatcctgacttcgatgtagtagctcgtgctgctgttcagatcaaaaatgcgattgatgcaacgattgaacttggcggagagaattatgtgttttggggtggtcgtgaaggctatatgtctcttctgaacacagatcagaaacgtgaaaaagaacaccttgcacagatgttgacgattgctcgtgactatgcccgtgcccgtggtttcaaaggtactttcctgatcgaaccgaaaccgatggaaccgactaaacatcaatatgacgtagatacggaaactgtaatcggcttcctgaaagctcatggtctggataaggatttcaaagtaaatatcgaggtgaatcacgcaactttggcaggtcacactttcgagcatgaattggctgtagctgtagacaatggtatgttgggctcaattgacgccaatcgtggtgactatcagaatggctgggatacagaccaattcccgatcgacaattatgaactgactcaggctatgatgcagattatccgtaatggtggtctcggtaccggtggtacgaactttgatgctaaaacccgtcgtaattctactgatctggaagatatctttattgctcacatcgcaggtatggacgctatggcccgtgcactcgaaagtgcagcggctctgctcgacgaatctccctataagaagatgctggctgaccgttatgcttcatttgatgggggcaaaggtaaagaatttgaagacggcaagctgactctggaggatgtggttgcttatgcaaaaacaaaaggcgaaccgaaacagactagcggcaagcaagaactttatgaggcaattctgaatatgtattgctaa

SEQ ID NO: 13 - protein, 442 aa, Parabacteroides distasonis
MSYFKGEKEFFPGIGQIQFEGRESKNPLAFHYYDADKVVMGKTLKDHLRFAMAYWHTLCAEGGDQFGGGTKTFPWNDSTDAITRAKYKMDAAFEFMTKCNIPYYCFHDVDVVDEAPTLGEFEKRLQTMVEHAKEHQAATGKKLLWSTANVFGHKRYMNGAATNPYFPTVACVGTQIKNAIDACIALGGENYVFWGGREGYMSLLNTNMKREKDHLAMMLTMARDYGRKNGFKGTFLIEPKPMEPTKHQYDVDSETVIGFLRHYGLDKDFALNIEVNHATLAGHTFEHELQAAADAGMLCSIDANRGDYQNGWDTDQFPMDIYELAQAWLVILEGGGLTTGGTNFDAKTRRNSTDLEDIFIAHIGGMDAFARALMIAADILENSDYRKMRAERYASFDAGEGKAFEDGKLTLEDLRTIALRDGEPKQISGKQELYEMIVNLHI

SEQ ID NO: 14 - DNA, 1329 bp, Parabacteroides_distasonis
atgtcttactttaagggtgaaaaagaattcttcccaggtatcggtcaaatccaatttgaaggtagagaatccaagaacccattggcttttcattattacgatgccgataaggttgtcatgggtaaaactttgaaggaccatttgagattcgctatggcttattggcatactttgtgtgctgaaggtggtgatcaatttggtggtggtacaaaaactttcccatggaatgattccaccgatgctattactagagccaagtacaaaatggatgctgcttttgaattcatgaccaagtgcaacattccttactactgcttccacgatgttgatgttgttgatgaagctccaactttgggtgaattcgaaaaaagattgcaaaccatggtcgaacatgccaaagaacatcaagctgctactggtaaaaagttgttgtggtctactgctaatgttttcggtcacaagagatatatgaacggtgctgctactaatccatactttccaactgttgcttgcgttggtactcaaatcaagaatgctattgatgcttgcattgctttgggtggtgaaaattatgttttctggggtggtagagaaggttacatgtctttgttgaacaccaacatgaagagagaaaaggatcatttggccatgatgttgactatggctagagattacggtagaaagaatggtttcaagggtactttcttgatcgaacctaaacctatggaacctactaagcaccaatacgatgttgattccgaaaccgttatcggtttcttgagacattacggtttggataaggatttcgccttgaacatcgaagttaaccatgctactttggctggtcatactttcgaacatgaattgcaagctgctgctgatgctggtatgttgtgttctattgatgctaacagaggtgactaccaaaatggttgggatactgatcaattcccaatggatatctacgaattggctcaagcttggttggttattttggaaggtggtggtttgactactggtggtactaattttgatgccaagaccagaagaaactccactgatttggaagacatcttcattgcccatatcggtggtatggatgcttttgctagagctttgatgattgctgccgatattttggaaaactccgactacagaaagatgagagctgaaagatacgcttcttttgatgctggtgaaggtaaggctttcgaagatggtaaattgaccttggaagatttgagaaccattgctttgagagatggtgaacctaagcaaatttccggtaagcaagaattatacgaaatgatcgtcaacttgcacatctaa

SEQ ID NO: 15 - protein, 437 aa, Cyllamyces aberensis
MVKEYFPAIQKIKFEGKDSKNPMAFHYYDAEKEIMGKKMKDWLRFAMAWWHTLCAEGSDQFGPGTKTFPWNEGTDPIEKAKQKVDAGFEIMTKLGIEHYCFHDVDLVDEGKNVEEYEKNLKTIVAYLKEKQKETGIKLLWSTANVFGHKRYMNGASTNPDFDVVARAIVQIKNAMDAGIELGAENYVFWGGREGYMSLLNTDQKREKEHMAMMLGLARDYARSKGFKGTFLIEPKPMEPTKHQYDVDTETVIGFLRAHGLDKDFKINIEVNHATLAGHTFEHELACAVDAGMLGSIDANRGDYQNGWDTDQFPIDQYELVQAWMEIIRGGGFTTGGTNFDAKTRRNSTDLEDIIIAHISGMDAMARALENAAKLLTESPYKKMKADRYASFDSGMGKDFEDGKLTFEQVYEYGKKVNEPKQTSGKQELYEAIVAMYM

SEQ ID NO: 16 - DNA, 1314 bp, Cyllamyces_aberensis
atggttaaggaatacttcccagctatccaaaagatcaagttcgaaggtaaggactctaagaacccaatggctttccactactacgacgctgaaaaggaaatcatgggtaagaagatgaaggactggttgagattcgctatggcttggtggcacactttgtgtgctgaaggttctgaccaattcggtccaggtactaagactttcccatggaacgaaggtactgacccaatcgaaaaggctaagcaaaaggttgacgctggtttcgaaatcatgactaagttgggtatcgaacactactgtttccacgacgttgacttggttgacgaaggtaagaacgttgaagaatacgaaaagaacttgaagactatcgttgcttacttgaaggaaaagcaaaaggaaactggtatcaagttgttgtggtctactgctaacgttttcggtcacaagagatacatgaacggtgcttctactaacccagacttcgacgttgttgctagagctatcgttcaaatcaagaacgctatggacgctggtatcgaattgggtgctgaaaactacgttttctggggtggtagagaaggttacatgtctttgttgaacactgaccaaaagagagaaaaggaacacatggctatgatgttgggtttggctagagactacgctagatctaagggtttcaagggtactttcttgatcgaaccaaagccaatggaaccaactaagcaccaatacgacgttgacactgaaactgttatcggtttcttgagagctcacggtttggacaaggacttcaagatcaacatcgaagttaaccacgctactttggctggtcacactttcgaacacgaattggcttgtgctgttgacgctggtatgttgggttctatcgacgctaacagaggtgactaccaaaacggttgggacactgaccaattcccaatcgaccaatacgaattggttcaagcttggatggaaatcatcagaggtggtggtttcactactggtggtactaacttcgacgctaagactagaagaaactctactgacttggaagacatcatcatcgctcacatctctggtatggacgctatggctagagctttggaaaacgctgctaagttgttgactgaatctccatacaagaagatgaaggctgacagatacgcttctttcgactctggtatgggtaaggacttcgaagacggtaagttgactttcgaacaagtttacgaatacggtaagaaggttaacgaaccaaagcaaacttctggtaagcaagaattgtacgaagctatcgttgctatgtacatgtga

SEQ ID NO: 17 - protein, 440 aa, Abiotrophia defectiva
MSELFQNIPKIKYEGANSKNPLAFHYYDAEKIVLGKTMKEHLPFAMAWWHNLCAAGTDMFGRDTADKSFGLEKGSMEHAKAKVDAGFEFMEKLGIKYFCFHDVDLVPEACDIKETNSRLDEISDYILEKMKGTDIKCLWGTANMFSNPRFVNGAGSTNSADVYCFAAAQIKKALDITVKLGGRGYVFWGGREGYETLLNTDVKFEQENIANLMKMAVEYGRSIGFKGDFYIEPKPKEPMKHQYDFDAATAIGFLRQYGLDKDFKLNIEANHATLAGHSFQHELRISSINGMLGSVDANQGDMLLGWDTDEFPFDVYDTTMCMYEVLKNGGLTGGFNFDAKNRRPSYTYEDMFYGFILGMDSFALGLIKAAKLIEEGTLDNFIKERYKSFESEIGKKIRSKSASLQELAAYAEEMGAPAMPGSGRQEYLQAALNQNLFGEV

SEQ ID NO: 18 - DNA, 1323 bp, Abiotrophia defectiva
atgtctgaattgttccaaaacatcccaaagatcaagtacgaaggtgctaactctaagaacccattggctttccactactacgacgctgaaaagatcgttttgggtaagactatgaaggaacacttgccattcgctatggcttggtggcacaacttgtgtgctgctggtactgacatgttcggtagagacactgctgacaagtctttcggtttggaaaagggttctatggaacacgctaaggctaaggttgacgctggtttcgaattcatggaaaagttgggtatcaagtacttctgtttccacgacgttgacttggttccagaagcttgtgacatcaaggaaactaactctagattggacgaaatctctgactacatcttggaaaagatgaagggtactgacatcaagtgtttgtggggtactgctaacatgttctctaacccaagattcgttaacggtgctggttctactaactctgctgacgtttactgtttcgctgctgctcaaatcaagaaggctttggacatcactgttaagttgggtggtagaggttacgttttctggggtggtagagaaggttacgaaactttgttgaacactgacgttaagttcgaacaagaaaacatcgctaacttgatgaagatggctgttgaatacggtagatctatcggtttcaagggtgacttctacatcgaaccaaagccaaaggaaccaatgaagcaccaatacgacttcgacgctgctactgctatcggtttcttgagacaatacggtttggacaaggacttcaagttgaacatcgaagctaaccacgctactttggctggtcactctttccaacacgaattgagaatctcttctatcaacggtatgttgggttctgttgacgctaaccaaggtgacatgttgttgggttgggacactgacgaattcccattcgacgtttacgacactactatgtgtatgtacgaagttttgaagaacggtggtttgactggtggtttcaacttcgacgctaagaacagaagaccatcttacacttacgaagacatgttctacggtttcatcttgggtatggactctttcgctttgggtttgatcaaggctgctaagttgatcgaagaaggtactttggacaacttcatcaaggaaagatacaagtctttcgaatctgaaatcggtaagaagatcagatctaagtctgcttctttgcaagaattggctgcttacgctgaagaaatgggtgctccagctatgccaggttctggtagacaagaatacttgcaagctgctttgaaccaaaacttgttcggtgaagtttga

SEQ ID NO: 19 - protein, 442 aa, Uncultured bacterium XYM2
MKLTVGDKEYFKGIKPIKFEGKDSDNPLAFKYYNPSQKVGKKTMEEHFRFAIAYWHTFCGTGGDPFGPGTKTFPWLQNSDAVQRAYDKMDAAFEFITKIGAPFYCFHDYDLVDEGPTLKESESRLQKVVDYAKKKQKASGVKLLWGTANLFSHPRYMNGAATNPDFDVVCYAASQVKNALDATIALGGANYVFWGGREGYMSLLNTNMKREQEHMAKFLHMAKDYARANGFKGTFFIEPKPMEPSKHQYDFDSATVIGFLRQFDLLGDFKLNIEVNHATLAHHTFQHELQVAADAGALGSIDANRGDYQNGWDTDQFPNNLYELAESMLVILEAGGFKSGGVNFDAKTRRNSTDLVDIFHAHIGGMDTFARSLLIAQAVLDNGEYTKIRKDRYSSFDSGKGKQFDQGKLSLEDLRNLAHKAGEPKQLSGKQEYIENLISRFI

SEQ ID NO: 20 - DNA, 1329 bp, Uncultured bacterium XYM2
atgaagttgaccgttggtgacaaagaatacttcaagggtattaagccaatcaagttcgaaggtaaggattccgataatccattggctttcaagtactacaacccatctcaaaaggttggtaaaaagaccatggaagaacatttcagattcgctattgcttactggcatactttttgtggtactggtggtgatccatttggtccaggtacaaaaacttttccatggttgcaaaactccgatgctgttcaaagagcttacgataagatggatgctgcctttgaattcattaccaaaattggtgctccattctactgcttccatgattacgatttggttgatgaaggtccaaccttgaaagaatccgaatccagattgcaaaaggtcgttgattacgctaagaaaaagcaaaaagcctccggtgttaagttgttgtggggtactgctaatttgttctcccatccaagatatatgaatggtgctgctacaaacccagatttcgatgttgtttgttatgctgcctctcaagttaagaatgctttggatgctactattgctttgggtggtgctaattatgttttttggggtggtagagaaggttacatgtctttgttgaacaccaacatgaagagagaacaagaacatatggctaagttcttgcatatggccaaggattatgctagagctaatggttttaagggtactttcttcatcgaacctaaacctatggaaccatctaagcaccaatacgattttgattccgctaccgttattggtttcttgagacaatttgatttgttgggtgacttcaagttgaacatcgaagttaaccatgctaccttggctcatcatacctttcaacatgaattgcaagttgctgctgatgctggtgctttaggttctattgatgctaatagaggtgactaccaaaacggttgggatactgatcaatttccaaacaacttgtacgaattggccgaatccatgttggttattttggaagctggtggttttaaatccggtggtgttaatttcgatgctaagaccagaagaaactctaccgatttggtcgatattttccatgctcatattggtggtatggatacctttgctagatccttgttgattgctcaagctgttttggataatggtgaatacaccaagatcagaaaggacagatactcctctttcgattctggtaaaggtaagcaattcgatcaaggtaaattgtccttggaagatttgagaaacttggctcacaaagctggtgaacctaagcaattgtctggtaagcaagaatatatcgaaaacttgatctccagattcatttga

SEQ ID NO: 21 - protein, 442 aa, Chitinophaga pinensis
MSITLGNQEYFKGIGKIAYEGPQSTNPFAYKWYDENRKIGGKTMKELFRFAVSYWHTFCGTGGDPFGPGTKAFPWLTATDAVQSAKDKMDAAFEFFTKLGVPYYCFHDVDLVDEGASISEYESRMQQIVEYAKEKQKASGVKLLWGTANVFSNPRYMNGAATNPDFAAVAYAGTQVKNSLDATIALGGENYVFWGGREGYMTLLNTDMKREQEHLARFLTMAKDYARKQGFTGTFFIEPKPCEPTKHQYDYDAATVIGFLRHFGLDKDFKLNLEVNHATLAGHTFQHELQVAADAGMLGSIDANRGDAQNGWDTDQFPMNLNDMVEFMLVILEAGGFSGGGVNFDAKTRRNSTDLEDIFHAHIGGIDSFARAAVIAEKVLEQSPYKQFRKDRYASFDSGKGKDFEAGTLTLEDLRSFAVSNGEPKHISGKQEWLENIINQYI

SEQ ID NO: 22 - DNA, 1329 bp, Chitinophaga pinensis
atgtccatcaccttgggtaatcaagaatacttcaagggtattggtaagattgcttacgaaggtccacaatctactaatccatttgcttacaagtggtacgacgaaaacagaaaaattggtggtaagaccatgaaggaattattcagattcgctgtttcctactggcatactttttgtggtactggtggtgatccatttggtccaggtacaaaagcttttccatggttgactgctactgatgctgttcaatctgctaaggataagatggatgctgcttttgaattcttcaccaaattgggtgttccttactactgcttccacgatgttgatttggttgatgaaggtgcttccatttctgaatacgaatccagaatgcaacaaatcgtcgaatacgccaaagaaaagcaaaaagcttccggtgttaagttgttgtggggtactgctaatgttttctccaacccaagatatatgaacggtgctgctactaatccagattttgctgctgttgcttatgctggtactcaagttaagaactctttggatgctaccattgctttgggtggtgaaaattatgttttctggggtggtagagaaggttacatgactttgttgaacaccgacatgaagagagaacaagaacatttggctagattcttgaccatggctaaagattacgctagaaagcaaggtttcaccggtacttttttcattgaacctaagccatgcgaacctaccaaacatcaatatgattacgatgctgccaccgttattggttttttgagacatttcggtttggacaaggacttcaagttgaacttggaagttaaccatgctactttggctggtcatactttccaacacgaattgcaagttgctgctgatgctggtatgttgggttctattgatgctaatagaggtgatgctcaaaacggttgggatactgatcaatttccaatgaacttgaacgacatggtcgaattcatgttggttattttggaagctggtggtttttctggtggtggtgttaattttgatgccaagactagaagaaactccaccgatttggaagatattttccatgctcatatcggtggtattgattcttttgctagagctgctgttatcgctgaaaaggttttggaacaatccccatacaagcaattcagaaaggatagatacgcttctttcgattctggtaagggtaaggattttgaagctggtactttgaccttggaagatttgagatctttcgctgtttctaacggtgaacctaaacatatttccggtaagcaagaatggttggaaaacatcatcaatcagtatatctaa

SEQ ID NO: 23 - protein, 439 aa, Prevotella ruminicola
MAKEYFPFTGKIPFEGKDSKNVMAFHYYEPEKVVMGKKMKDWLKFAMAWWHTLGGASADQFGGQTRSYEWDKAADAVQRAKDKMDAGFEIMDKLGIEYFCFHDVDLVEEGETIAEYERRMKEITDYALVKMKEYPNIKLLWGTANVFGNKRYANGASTNPDFDVVARAIVQIKNAIDATIKLGGTNYVFWGGREGYMSLLNTDQKREKEHMATMLTMARDYARAKGFKGTFLIEPKPMEPSKHQYDVDTETVCGFLRAHGLDKDFKVNIEVNHATLAGHTFEHELACAVDNGMLGSIDANRGDAQNGWDTDQFPIDNFELTQAMLEIIRNGGLGNGGTNFDAKIRRNSTDLEDLFIAHISGMDAMARALMNAAAILEESELPKMKKERYASFDNGIGKDFEDGKLTLEQAYEYGKKVEEPKQTSGKQEKYETTVALYCK

SEQ ID NO: 24 - DNA, 1320 bp, Prevotella ruminicola
atggctaaggaatacttcccattcactggtaagatcccattcgaaggtaaggactctaagaacgttatggctttccactactacgaaccagaaaaggttgttatgggtaagaagatgaaggactggttgaagttcgctatggcttggtggcacactttgggtggtgcttctgctgaccaattcggtggtcaaactagatcttacgaatgggacaaggctgctgacgctgttcaaagagctaaggacaagatggacgctggtttcgaaatcatggacaagttgggtatcgaatacttctgtttccacgacgttgacttggttgaagaaggtgaaactatcgctgaatacgaaagaagaatgaaggaaatcactgactacgctttggttaagatgaaggaatacccaaacatcaagttgttgtggggtactgctaacgttttcggtaacaagagatacgctaacggtgcttctactaacccagacttcgacgttgttgctagagctatcgttcaaatcaagaacgctatcgacgctactatcaagttgggtggtactaactacgttttctggggtggtagagaaggttacatgtctttgttgaacactgaccaaaagagagaaaaggaacacatggctactatgttgactatggctagagactacgctagagctaagggtttcaagggtactttcttgatcgaaccaaagccaatggaaccatctaagcaccaatacgacgttgacactgaaactgtttgtggtttcttgagagctcacggtttggacaaggacttcaaggttaacatcgaagttaaccacgctactttggctggtcacactttcgaacacgaattggcttgtgctgttgacaacggtatgttgggttctatcgacgctaacagaggtgacgctcaaaacggttgggacactgaccaattcccaatcgacaacttcgaattgactcaagctatgttggaaatcatcagaaacggtggtttgggtaacggtggtactaacttcgacgctaagatcagaagaaactctactgacttggaagacttgttcatcgctcacatctctggtatggacgctatggctagagctttgatgaacgctgctgctatcttggaagaatctgaattgccaaagatgaagaaggaaagatacgcttctttcgacaacggtatcggtaaggacttcgaagacggtaagttgactttggaacaagcttacgaatacggtaagaaggttgaagaaccaaagcaaacttctggtaagcaagaaaagtacgaaactactgttgctttgtactgtaagtga

SEQ ID NO: 25 - protein, 437 aa, Piromyces equi
MAKEYFPQIQKIKFEGKDSKNPLAFHYYDAEKEVMGKKMKDWLRFAMAWWHTLCAEGADQFGGGTKSFPWNEGTDAIEIAKQKVDAGFEIMQKLGIPYYCFHDVDLVSEGNSIEEYESNLKAVVAYLKEKQKETGIKLLWSTANVFGHKRYMNGASTNPDFDVVARAIVQIKNAIDAGIELGAENYVFWGGREGYMSLLNTDQKREKEHMATMLTMARDYARSKGFKGTFLIEPKPMEPTKHQYDVDTETAIGFLKAHNLDKDFKVNIEVNHATLAGHTFEHELACAVDAGMLGSIDANRGDYQNGWDTDQFPIDQYELVQAWMEIIRGGGFVTGGTNFDAKTRRNSTDLEDIIIAHVSGMDAMARALENAAKLLQESPYTKMKKERYASFDSGIGKDFEDGKLTLEQVYEYGKKNGEPKQTSGKQELYEAIVAMYQ

SEQ ID NO: 26 - DNA, 1314 bp, Piromyces equi
atggccaaagaatacttcccacaaatccaaaagatcaagttcgaaggtaaggactctaagaatccattggctttccattactacgacgccgaaaaagaagttatgggtaagaaaatgaaggactggttgagatttgctatggcttggtggcatactttgtgtgctgaaggtgctgatcaatttggtggtggtacaaaatctttcccatggaatgaaggtactgatgccattgaaattgccaagcaaaaagttgatgccggtttcgaaattatgcaaaagttgggtattccttactactgcttccacgatgttgatttggtttctgaaggtaactccatcgaagaatacgaatctaacttgaaggctgttgtcgcctacttgaaagaaaaacaaaaagaaaccggtattaagttgttgtggtctaccgctaatgttttcggtcacaagagatatatgaacggtgcttctactaatccagatttcgatgttgttgctagagccatcgttcaaatcaagaatgctattgatgctggtattgaattgggtgccgaaaattatgttttttggggtggtagagaaggttacatgtctttgttgaacaccgatcaaaaaagagaaaaagaacacatggctaccatgttgactatggctagagattacgctagatctaagggttttaagggtactttcttgatcgaacctaaacctatggaacctactaagcaccaatatgatgttgataccgaaaccgctatcggttttttgaaggctcataacttggataaggacttcaaggttaacatcgaagtcaaccatgctactttggctggtcatacttttgaacatgaattggcttgtgctgttgacgcaggtatgttgggttcaattgatgctaatagaggtgactaccaaaacggttgggatacagatcaattcccaatcgatcaatacgaattggttcaagcttggatggaaattatcagaggtggtggttttgttaccggtggtactaattttgatgccaagactagaagaaactccaccgatttggaagatatcattatcgctcatgtttccggtatggatgctatggcaagagctttggaaaatgctgctaagttgttacaagaatccccatacaccaagatgaagaaagaaagatacgcctctttcgattccggtattggtaaggattttgaagatggtaaattgaccttggaacaagtctacgaatacggtaaaaagaacggtgaacctaagcaaacttctggtaagcaagaattatacgaagctatcgttgccatgtaccaatga

SEQ ID NO: 27 - protein, 438 aa, Clostridium phytofermentans
MKNYFPNVPEVKYEGPNSTNPFAFKYYDANKVVAGKTMKEHCRFALSWWHTLCAGGADPFGVTTMDRTYGNITDPMELAKAKVDAGFELMTKLGIEFFCFHDADIAPEGDTFEESKKNLFEIVDYIKEKMDQTGIKLLWGTANNFSHPRFMHGASTSCNADVFAYAAAKIKNALDATIKLGGKGYVFWGGREGYETLLNTDLGLELDNMARLMKMAVEYGRANGFDGDFYIEPKPKEPTKHQYDFDTATVLAFLRKYGLEKDFKMNIEANHATLAGHTFEHELAMARVNGAFGSVDANQGDPNLGWDTDQFPTDVHSATLAMLEVLKAGGFTNGGLNFDAKVRRGSFEFDDIAYGYIAGMDTFALGLIKAAEIIDDGRIAKFVDDRYASYKTGIGKAIVDGTTSLEELEQYVLTHSEPVMQSGRQEVLETIVNNILFR

SEQ ID NO: 28 - DNA, 1317 bp, Clostridium phytofermentans
atgaagaactacttcccaaacgttccagaagttaagtacgaaggtccaaactctactaatccattcgctttcaagtactacgatgccaacaaagttgttgctggtaagactatgaaggaacattgcagatttgctttgtcttggtggcatactttgtgtgctggtggtgctgatccatttggtgttactactatggatagaacctacggtaacattaccgatccaatggaattggctaaagctaaagttgatgccggttttgaattgatgaccaagttgggtattgaattcttctgcttccatgatgctgatattgctccagaaggtgatactttcgaagaatccaagaagaacttgttcgaaatcgtcgactacatcaaagaaaagatggatcaaaccggtatcaagttgttgtggggtactgctaacaatttctctcatccaagattcatgcatggtgcttctacatcttgtaacgctgatgtttttgcttatgctgctgccaagattaagaatgctttggatgctactattaagttgggtggtaagggttatgttttttggggtggtagagaaggttacgaaaccttgttgaatactgacttgggtttggaattggataacatggctagattgatgaagatggcagttgaatacggtagagctaatggttttgatggtgatttctacatcgaacctaagccaaaagaacctactaagcaccaatacgattttgatactgctaccgttttggccttcttgagaaagtatggtttggaaaaggacttcaagatgaacatcgaagctaaccatgctactttggctggtcatacttttgaacatgaattggcaatggctagagttaatggtgcttttggttctgttgatgccaatcaaggtgatcctaatttgggttgggatactgatcaatttccaaccgatgttcactctgctactttagctatgttggaagttttgaaggctggtggttttactaatggtggtttgaatttcgatgccaaggttagaagaggttcctttgaatttgacgatattgcttacggttacattgctggtatggatacttttgctttgggtttgattaaggccgccgaaattattgatgatggtagaattgctaagttcgttgatgatagatacgcctcttacaagactggtattggtaaagcaatcgttgatggtactacctccttggaagaattggaacaatatgttttgacccactccgaaccagttatgcaatctggtagacaagaagttttggaaaccatcgtcaacaatattttgtttagatga

SEQ ID NO: 29 - protein, 165 aa, Saccharomyces cerevisiae
MLPVITRFARPALMAIRPVNAMGVLRATSITKRLYHPKVIEHYTHPRNVGSLDKKLPNVGTGLVGAPACGDVMRLQIKVNDSTGVIEDVKFKTFGCGSAIASSSYMTELVQGMTLDDAAKIKNTEIAKELSLPPVKLHCSMLAEDAIKAAIKDYKSKRNTPTMLS

SEQ ID NO: 30 - DNA, 498 bp, Saccharomyces cerevisiae
atgcttcctgttataacgagatttgcaaggcctgctctgatggccatcagacctgtgaatgccatgggggttttgagagcgaccagcataacgaaaaggctttatcatcccaaggtcatagagcattatacacatccaagaaacgtcggctcattagataaaaaattgcccaacgtcggcactggtctagtgggtgcgccagcgtgcggtgatgtgatgaggttgcagatcaaagtcaacgactctactggcgttattgaagatgtcaaattcaagacttttggatgtggctccgccattgcctcctcttcatatatgactgaattggtacaggggatgaccttggacgatgcggcaaaaattaagaacactgaaattgctaaggagttgagcttgcccccagtcaagttgcattgctctatgttagcagaagatgcgatcaaggcagctattaaggactacaaatctaagagaaacactccaaccatgttatcgtaa

SEQ ID NO: 31 - protein, 174 aa, Saccharomyces cerevisiae
MIKRSLASLVRVSSVMGRRYMIAAAGGERARFCPAVTNKKNHTVNTFQKRFVESSTDGQVVPQEVLNLPLEKYHEEADDYLDHLLDSLEELSEAHPDCIPDVELSHGVMTLEIPAFGTYVINKQPPNKQIWLASPLSGPNRFDLLNGEWVSLRNGTKLTDILTEEVEKAISKSQ

SEQ ID NO: 32 - DNA, 525 bp, Saccharomyces cerevisiae
atgattaagcggtctctcgcaagtttagttcgagtcagctctgtaatgggcagaagatatatgatagcagcggcaggaggagaacgtgccagattttgtccagctgtaacaaataaaaagaatcatactgtaaatacttttcagaagagatttgtagaatcctcgacagatggtcaagttgtgcctcaagaagtgttaaacttaccgcttgaaaaataccatgaagaggcagatgactacctagaccatttactagatagcttagaagaactgagtgaggctcatccggactgtatacctgatgtagagctaagccatggcgtaatgacattggaaattccagcttttggaacgtatgtaataaacaaacagcctccaaataagcaaatttggctggcatcaccattgtccgggcctaacagatttgaccttctcaatggggagtgggtttcgttaagaaatggcacaaagctaacagatatacttactgaagaagttgagaaggccatttctaaaagccaataa

SEQ ID NO: 33 - protein, 497 aa, Saccharomyces cerevisiae
MLKSTATRSITRLSQVYNVPAATYRACLVSRRFYSPPAAGVKLDDNFSLETHTDIQAAAKAQASARASASGTTPDAVVASGSTAMSHAYQENTGFGTRPIYLDMQATTPTDPRVLDTMLKFYTGLYGNPHSNTHSYGWETNTAVENARAHVAKMINADPKEIIFTSGATESNNMVLKGVPRFYKKTKKHIITTRTEHKCVLEAARAMMKEGFEVTFLNVDDQGLIDLKELEDAIRPDTCLVSVMAVNNEIGVIQPIKEIGAICRKNKIYFHTDAAQAYGKIHIDVNEMNIDLLSISSHKIYGPKGIGATYVRRRPRVRLEPLLSGGGQERGLRSGTLAPPLVAGFGEAARLMKKEFDNDQAHIKRLSDKLVKGLLSAEHTTLNGSPDHRYPGCVNVSFAYVEGESLLMALRDIALSSGSACTSASLEPSYVLHALGKDDALAHSSIRFGIGRFSTEEEVDYVVKAVSDRVKFLRELSPLWEMVQEGIDLNSIKWSGH

SEQ ID NO: 34 - DNA, 1494 bp, Saccharomyces cerevisiae
atgttgaaatcaactgctacaagatcgataacaagattatctcaagtttacaacgttccagcggccacatatagggcttgtttggtaagcaggagattctattcccctcctgcagcaggcgtgaagttagacgacaacttctctctggaaacgcataccgatattcaggctgctgcaaaggcacaggctagtgcccgtgcgagtgcatccggtaccaccccagatgctgtagtagcttctggtagcactgcaatgagccatgcttatcaagaaaacacaggttttggtactcgtcccatatatcttgacatgcaagccactacaccaacagaccctagggttttggatacgatgttgaagttttatacgggactttatggtaatcctcattccaacactcactcttacggttgggaaacaaatactgctgtggaaaatgctagagctcacgtagcaaagatgatcaatgccgaccccaaggaaataatattcacttcgggagcgaccgaatctaataatatggttcttaagggtgtcccaagattttataagaagactaagaaacacatcatcaccactagaacggaacacaagtgtgtcttggaagccgcacgggccatgatgaaggagggatttgaagtcactttcctaaatgtggacgatcaaggtcttatcgatttgaaggaattggaagatgccattagaccagatacctgtctcgtctctgtgatggctgtcaataatgaaatcggtgtcattcaacctattaaagaaattggtgcaatttgtagaaagaataagatctactttcataccgacgccgcacaagcctatggtaagattcacattgatgtcaatgaaatgaacattgatttactatcaatttcttctcacaagatttacggtccaaagggaataggtgccacctatgtaagaaggagaccaagagttagattagaacctttactatccggtggtggccaagagagaggattgagatctggtactttggcccccccattggtagcgggatttggtgaagctgcgagattgatgaagaaagaatttgacaacgaccaagctcacatcaaaagactatccgataaattagtcaaaggtctattatccgctgaacataccacgttgaacggatctccagatcatcgttatccagggtgtgttaacgtttctttcgcctacgtggaaggagaatctttattgatggcactaagggatatcgcattatcctcgggttcagcctgtacatctgcttccctagaaccttcttatgttttacatgcgctgggtaaggatgatgcattagcccattcttccatcagatttggtattggtagatttagtactgaagaggaggtcgactacgtcgttaaggccgtttctgacagagtaaaattcttgagggaactttcaccattatgggaaatggttcaagaaggtattgacttaaactccatcaaatggtcaggtcattga

SEQ ID NO: 35 - protein, 438 aa, Artificial Sequence
  CX386 chimeric xylose isomerase
MAKEYFPFTGKIPFEGKDSKNVMAFHYYEPEKVVMGKKMKDWLKFAMAWWHTLGGASADQFGGQTRSYEWDKAADAVQRAKDKMDAGFEIMDKLGIEYFCFHDVDLVEEGETIAEYERRMKEITDYALVKMKEYPNIKLLWGTANVFSNPRYMNGAATNPDFAAVAYAGTQVKNSLDATIALGGENYVFWGGREGYMSLLNTNMKREKDHLAMMLTMARDYGRKNGFKGTFLIEPKPMEPTKHQYDVDSETVIGFLRHYGLDKDFALNIEVNHATLAGHTFEHELQAAADAGMLCSIDANRGDYQNGWDTDQFPMDIYELAQAWLVILEGGGLTTGGTNFDAKTRRNSTDLEDIFIAHIGGMDAFARALMIAADILENSDYRKMRAERYASFDAGEGKAFEDGKLTLEDLRTIALRDGEPKQISGKQELYEMIVNLHI

SEQ ID NO: 36 - DNA, 1317 bp, Artificial Sequence
  CX386 chimeric xylose isomerase
atggctaaggaatacttcccattcactggtaagatcccattcgaaggtaaggactctaagaacgttatggctttccactactacgaaccagaaaaggttgttatgggtaagaagatgaaggactggttgaagttcgctatggcttggtggcacactttgggtggtgcttctgctgaccaattcggtggtcaaactagatcttacgaatgggacaaggctgctgacgctgttcaaagagctaaggacaagatggacgctggtttcgaaatcatggacaagttgggtatcgaatacttctgtttccacgacgttgacttggttgaagaaggtgaaactatcgctgaatacgaaagaagaatgaaggaaatcactgactacgctttggttaagatgaaggaatacccaaacatcaagttgttgtggggtactgctaatgttttctccaacccaagatatatgaacggtgctgctactaatccagattttgctgctgttgcttatgctggtactcaagttaagaactctttggatgctaccattgctttgggtggtgaaaattatgttttctggggtggtagagaaggttacatgtctttgttgaacaccaacatgaagagagaaaaggatcatttggccatgatgttgactatggctagagattacggtagaaagaatggtttcaagggtactttcttgatcgaacctaaacctatggaacctactaagcaccaatacgatgttgattccgaaaccgttatcggtttcttgagacattacggtttggataaggatttcgccttgaacatcgaagttaaccatgctactttggctggtcatactttcgaacatgaattgcaagctgctgctgatgctggtatgttgtgttctattgatgctaacagaggtgactaccaaaatggttgggatactgatcaattcccaatggatatctacgaattggctcaagcttggttggttattttggaaggtggtggtttgactactggtggtactaattttgatgccaagaccagaagaaactccactgatttggaagacatcttcattgcccatatcggtggtatggatgcttttgctagagctttgatgattgctgccgatattttggaaaactccgactacagaaagatgagagctgaaagatacgcttcttttgatgctggtgaaggtaaggctttcgaagatggtaaattgaccttggaagatttgagaaccattgctttgagagatggtgaacctaagcaaatttccggtaagcaagaattatacgaaatgatcgtcaacttgcacatctaa

SEQ ID NO: 37 - protein, 438 aa, Artificial Sequence
  CX1224 chimeric xylose isomerase
MTKEYFPFTGKIPYEGKDSNNVMAFHYYEPEKVVMGKKMKDWLKFAMAWWHTLGGASADQFGGQTRSYEWDKAADAVQRAKDKMDAGFEIMDKLGIEYFCFHDVDLVEEGETIAEYERRMKEITDYALVKMKEYPNIKLLWGTANVFSNPRYMNGAATNPDFAAVAYAGTQVKNSLDATIALGGENYVFWGGREGYMSLLNTNMKREKDHLAMMLTMARDYGRKNGFKGTFLIEPKPMEPTKHQYDVDSETVIGFLRHYGLDKDFALNIEVNHATLAGHTFEHELQAAADAGMLCSIDANRGDYQNGWDTDQFPMDIYELAQAWLVILENGGLTTGGTNFDAKTRRNSTDLEDIFIAHIGGMDAFARALMIAADILENSDYRKMRAERYGTFDAGEGKAFEEGQLTLEDLRTIALRDGDPKKISGKQELYEMIVNLHI

SEQ ID NO: 38 - DNA, 1317 bp, Artificial Sequence
  CX1224 chimeric xylose isomerase
atgactaaggaatacttcccattcactggtaagatcccatacgaaggtaaggactctaataacgttatggctttccactactacgaaccagaaaaggttgttatgggtaagaagatgaaggactggttgaagttcgctatggcttggtggcacactttgggtggtgcttctgctgaccaattcggtggtcaaactagatcttacgaatgggacaaggctgctgacgctgttcaaagagctaaggacaagatggacgctggtttcgaaatcatggacaagttgggtatcgaatacttctgtttccacgacgttgacttggttgaagaaggtgaaactatcgctgaatacgaaagaagaatgaaggaaatcactgactacgctttggttaagatgaaggaatacccaaacatcaagttgttgtggggtactgctaatgttttctccaacccaagatatatgaacggtgctgctactaatccagattttgctgctgttgcttatgctggtactcaagttaagaactctttggatgctaccattgctttgggtggtgaaaattatgttttctggggtggtagagaaggttacatgtctttgttgaacaccaacatgaagagagaaaaggatcatttggccatgatgttgactatggctagagattacggtagaaagaatggtttcaagggtactttcttgatcgaacctaaacctatggaacctactaagcaccaatacgatgttgattccgaaaccgttatcggtttcttgagacattacggtttggataaggatttcgccttgaacatcgaagttaaccatgctactttggctggtcatactttcgaacatgaattgcaagctgctgctgatgctggtatgttgtgttctattgatgctaacagaggtgactaccaaaatggttgggatactgatcaattcccaatggatatctacgaattggctcaagcttggttggttattttggaaaacggtggtttgactactggtggtactaattttgatgccaagaccagaagaaactccactgatttggaagacatcttcattgcccatatcggtggtatggatgcttttgctagagctttgatgattgctgccgatattttggaaaactccgactacagaaagatgagagctgaaagatacggtacttttgatgctggtgaaggtaaggctttcgaagaaggtcaattgaccttggaagatttgagaaccattgctttgagagatggtgatcctaagaagatttccggtaagcaagaattatacgaaatgatcgtcaacttgcacatctaa

SEQ ID NO: 39 - protein, 457 aa, Lachnoanaerobaculum_saburreum
MKTKNNIICTIALKGDIFMKEFFPGISPVKFEGRDSKNPLSFKYYDAKRVIMGKTMEEHLSFAMAWWHNLCACGVDMFGQGTVDKSFGESSGTMEHARAKVDAGIEFMKKLGIKYYCFHDTDIVPEDQEDINVTNARLDEITDYILEKTKDTDIKCLWTTCNMFSNPRFMNGAGSSNSADVFCFAAAQAKKGLENAVKLGAKGFVFWGGREGYETLLNTDMKLEEENIATLFTMCRDYGRSIGFMGDFYIEPKPKEPMKHQYDFDAATAIGFLRKYGLDKDFKLNIEANHATLAGHTFQHELRVCAVNGMMGSVDANQGDTLLGWDTDQFPTNVYDTTLAMYEILKAGGLRGGLNFDSKNRRPSNTADDMFYGFIAGMDTFALGLIKAAEIIEDGRIDDFVKERYASYNSGIGKKIRNRKVTLIECAEYAAKLKKPELPESGRQEYLESVVNNILFG

SEQ ID NO: 40 - DNA, 1374 bp, Lachnoanaerobaculum_saburreum
atgaagactaagaacaacatcatctgtactatcgctttgaagggtgacatcttcatgaaggaattcttcccaggtatctctccagttaagttcgaaggtagagactctaagaacccattgtctttcaagtactacgacgctaagagagttatcatgggtaagactatggaagaacacttgtctttcgctatggcttggtggcacaacttgtgtgcttgtggtgttgacatgttcggtcaaggtactgttgacaagtctttcggtgaatcttctggtactatggaacacgctagagctaaggttgacgctggtatcgaattcatgaagaagttgggtatcaagtactactgtttccacgacactgacatcgttccagaagaccaagaagacatcaacgttactaacgctagattggacgaaatcactgactacatcttggaaaagactaaggacactgacatcaagtgtttgtggactacttgtaacatgttctctaacccaagattcatgaacggtgctggttcttctaactctgctgacgttttctgtttcgctgctgctcaagctaagaagggtttggaaaacgctgttaagttgggtgctaagggtttcgttttctggggtggtagagaaggttacgaaactttgttgaacactgacatgaagttggaagaagaaaacatcgctactttgttcactatgtgtagagactacggtagatctatcggtttcatgggtgacttctacatcgaaccaaagccaaaggaaccaatgaagcaccaatacgacttcgacgctgctactgctatcggtttcttgagaaagtacggtttggacaaggacttcaagttgaacatcgaagctaaccacgctactttggctggtcacactttccaacacgaattgagagtttgtgctgttaacggtatgatgggttctgttgacgctaaccaaggtgacactttgttgggttgggacactgaccaattcccaactaacgtttacgacactactttggctatgtacgaaatcttgaaggctggtggtttgagaggtggtttgaacttcgactctaagaacagaagaccatctaacactgctgacgacatgttctacggtttcatcgctggtatggacactttcgctttgggtttgatcaaggctgctgaaatcatcgaagacggtagaatcgacgacttcgttaaggaaagatacgcttcttacaactctggtatcggtaagaagatcagaaacagaaaggttactttgatcgaatgtgctgaatacgctgctaagttgaagaagccagaattgccagaatctggtagacaagaatacttggaatctgttgttaacaacatcttgttcggttga

SEQ ID NO: 41 - protein, 439 aa, Lactobacillus_xylosus
MAYFNDIAPIKYEGTKTKNMFAFRHYNPEEVVAGKTMEEQLHFALAFWHTITMDGSDPFGGATMERPWDLEGGSELDRAHRRVDAFFEIAEKLGVKYYCFHDIDIAPTGNSLKEFYANLDEITDHLLEKQKATGIKLLWNTANMFSNPRYMNGVSTSNRAEVFAYGAAQVKKGLELSKKLGGENYVFWGGREGYESLLNTDMGLEMDHMAKFFHLAIDYAKSINHLPIFLIEPKPKEPMTHQYDFDSATALAFLQKYDLDKYFKLNLETNHAWLAGHTFEHELNTARTFNALGSIDANQGNYLLGWDTDEFPTLVIDITLAMHQILLNGGLGKGGINFDAKVRRTSFKAEDLILAHIAGMDTYARALKGAAAIIEDKFLSDIVDERYSSYRNTEVGQSIENGTATFESLAAFALEYGDDIELDSNHLEYIKSVLNDYLV

SEQ ID NO: 42 - DNA, 1320 bp, Lactobacillus_xylosus
atggcttacttcaacgacatcgctccaatcaagtacgaaggtactaagactaagaacatgttcgctttcagacactacaacccagaagaagttgttgctggtaagactatggaagaacaattgcacttcgctttggctttctggcacactatcactatggacggttctgacccattcggtggtgctactatggaaagaccatgggacttggaaggtggttctgaattggacagagctcacagaagagttgacgctttcttcgaaatcgctgaaaagttgggtgttaagtactactgtttccacgacatcgacatcgctccaactggtaactctttgaaggaattctacgctaacttggacgaaatcactgaccacttgttggaaaagcaaaaggctactggtatcaagttgttgtggaacactgctaacatgttctctaacccaagatacatgaacggtgtttctacttctaacagagctgaagttttcgcttacggtgctgctcaagttaagaagggtttggaattgtctaagaagttgggtggtgaaaactacgttttctggggtggtagagaaggttacgaatctttgttgaacactgacatgggtttggaaatggaccacatggctaagttcttccacttggctatcgactacgctaagtctatcaaccacttgccaatcttcttgatcgaaccaaagccaaaggaaccaatgactcaccaatacgacttcgactctgctactgctttggctttcttgcaaaagtacgacttggacaagtacttcaagttgaacttggaaactaaccacgcttggttggctggtcacactttcgaacacgaattgaacactgctagaactttcaacgctttgggttctatcgacgctaaccaaggtaactacttgttgggttgggacactgacgaattcccaactttggttatcgacatcactttggctatgcaccaaatcttgttgaacggtggtttgggtaagggtggtatcaacttcgacgctaaggttagaagaacttctttcaaggctgaagacttgatcttggctcacatcgctggtatggacacttacgctagagctttgaagggtgctgctgctatcatcgaagacaagttcttgtctgacatcgttgacgaaagatactcttcttacagaaacactgaagttggtcaatctatcgaaaacggtactgctactttcgaatctttggctgctttcgctttggaatacggtgacgacatcgaattggactctaaccacttggaatacatcaagtctgttttgaacgactacttggtttga